European Patent Application EP 4 353 831 A1, published April 17, 2024. Title: PRODUCT AND METHOD FOR ANALYZING OMICS INFORMATION OF SAMPLE. Applicant: OCEAN UNIVERSITY OF CHINA. The sequence listing filed with the application follows.

SEQUENCE LISTING (15 sequences)

SEQ ID NO: 1 - DNA, 15 bp, Artificial Sequence
  The first binding domain of an adapter
aggccagagcattcg

SEQ ID NO: 2 - DNA, 15 bp, Artificial Sequence
  The second binding domain of an adapter; primer 4
atccacgtgcttgag

SEQ ID NO: 3 - DNA, 24 bp, Artificial Sequence
  The amplification primer recognition sequence; primer 2; primer 3, primer 8
ccctacacgacgctcttccgatct

SEQ ID NO: 4 - DNA, 30 bp, Artificial Sequence
  The oligonucleotide adapter
cgaatgctctggcctctcaagcacgtggat

SEQ ID NO: 5 - DNA, 23 bp, Artificial Sequence
  Primer 1
aagcagtggtatcaacgcagagt

SEQ ID NO: 6 - DNA, 22 bp, Artificial Sequence
  Primer 5
gtggtatcaacgcagagtgatc

SEQ ID NO: 7 - DNA, 17 bp, Artificial Sequence
  Primer 6
cttccgatctggtctcg

SEQ ID NO: 8 - DNA, 22 bp, Artificial Sequence
  Primer 7
cagacgtgtgctcttccgatct

SEQ ID NO: 9 - DNA, 22 bp, Artificial Sequence
  Probe
agatcggaagagcacacgtctg

SEQ ID NO: 10 - DNA, 34 bp, Artificial Sequence
  Probe for epigenomic analysis
aggccagagcattcgagatgtgtataagagacag

SEQ ID NO: 11 - DNA, 34 bp, Artificial Sequence
  Tn5B primer
gtctcgtgggctcggagatgtgtataagagacag

SEQ ID NO: 12 - DNA, 19 bp, Artificial Sequence
  Tn5M primer
ctgtctcttatacacatct

SEQ ID NO: 13 - DNA, 34 bp, Artificial Sequence
  The 3’ end sequence of the antibody probe
ctgtctcttatacacatctccgagcccacgagac

SEQ ID NO: 14 - DNA, 30 bp, Artificial Sequence
  The chain conversion primer
aagcagtggtatcaacgcagagtacatggg

SEQ ID NO: 15 - DNA, 22 bp, Artificial Sequence
  Downstream sequence
gatcactctgcgttgataccac